European Patent Application EP 4 194 007 A1, published June 14, 2023. Title: Conjugate vaccine which targets an endogenous protein involving disease. Applicant: Osaka University. The sequence listing filed with the application follows.

SEQUENCE LISTING (41 sequences)

SEQ ID NO: 1 - protein, 20 aa, synthetic construct
  REGION 1..20: note = synthesized peptide
ELKLIFLHRLKRLRKRLKRK

SEQ ID NO: 2 - protein, 9 aa, Homo sapiens
ENSTFDEFG

SEQ ID NO: 3 - protein, 9 aa, Homo sapiens
NKRQLITEE

SEQ ID NO: 4 - protein, 10 aa, Homo sapiens
KNTYRLKLYS

SEQ ID NO: 5 - protein, 10 aa, Homo sapiens
YSDESLQYPK

SEQ ID NO: 6 - protein, 10 aa, Homo sapiens
PPHFDKSKKY

SEQ ID NO: 7 - protein, 10 aa, Homo sapiens
GLPTPEDNLD

SEQ ID NO: 8 - protein, 9 aa, Homo sapiens
FSKEAKYYQ

SEQ ID NO: 9 - protein, 15 aa, Homo sapiens
NSSVFLENSTFDEFG

SEQ ID NO: 10 - protein, 8 aa, Homo sapiens
RSSDYYNR

SEQ ID NO: 11 - protein, 15 aa, Homo sapiens
PKRSSDYYNRSTSPW

SEQ ID NO: 12 - protein, 11 aa, Homo sapiens
YQCRVTHPHLP

SEQ ID NO: 13 - protein, 10 aa, Homo sapiens
GHHHKPGLGE

SEQ ID NO: 14 - protein, 10 aa, Homo sapiens
LRPRGQPNQC

SEQ ID NO: 15 - protein, 9 aa, Homo sapiens
SRHLAQASQ

SEQ ID NO: 16 - protein, 10 aa, Homo sapiens
SRSGKRRGER

SEQ ID NO: 17 - protein, 9 aa, Mus musculus
ENSTFESFG

SEQ ID NO: 18 - protein, 10 aa, Mus musculus
KSTFRVKSYS

SEQ ID NO: 19 - protein, 10 aa, Mus musculus
GLPIPEDNLD

SEQ ID NO: 20 - protein, 15 aa, Mus musculus
NSSIFLENSTFESFG

SEQ ID NO: 21 - protein, 8 aa, Mus musculus
RPSDYLNR

SEQ ID NO: 22 - protein, 15 aa, Mus musculus
SRRPSDYLNRSTSPW

SEQ ID NO: 23 - protein, 11 aa, Mus musculus
YQCIVDHPDFP

SEQ ID NO: 24 - protein, 10 aa, Mus musculus
GHSHGKGCGK

SEQ ID NO: 25 - protein, 10 aa, Mus musculus
PALRSRRQPG

SEQ ID NO: 26 - protein, 9 aa, Mus musculus
CRSRPSAKA

SEQ ID NO: 27 - protein, 10 aa, Mus musculus
SFSRSGRRRG

SEQ ID NO: 28 - protein, 9 aa, Mus musculus
RMFPNAPYL

SEQ ID NO: 29 - protein, 11 aa, Homo sapiens
CPNSEDKNFPR

SEQ ID NO: 30 - protein, 10 aa, Homo sapiens
RNEDPERYPS

SEQ ID NO: 31 - protein, 7 aa, Homo sapiens
NRSTSPW

SEQ ID NO: 32 - protein, 7 aa, Homo sapiens
LHRNEDP

SEQ ID NO: 33 - protein, 9 aa, Homo sapiens
RYPSVIWEA

SEQ ID NO: 34 - protein, 10 aa, Homo sapiens
PKRSSDYYNR

SEQ ID NO: 35 - protein, 12 aa, Homo sapiens
TNPKRSSDYYNR

SEQ ID NO: 36 - protein, 14 aa, Homo sapiens
TNTNPKRSSDYYNR

SEQ ID NO: 37 - protein, 11 aa, Mus musculus
CPNTEAKDFLQ

SEQ ID NO: 38 - protein, 10 aa, Mus musculus
RNEDPDRYPS

SEQ ID NO: 39 - protein, 10 aa, Mus musculus
SRRPSDYLNR

SEQ ID NO: 40 - protein, 12 aa, Mus musculus
VSSRRPSDYLNR

SEQ ID NO: 41 - protein, 14 aa, Mus musculus
AKVSSRRPSDYLNR